European Patent Application EP 4 491 714 A2, published January 15, 2025. Title: Transglutaminase Mediated High Molecular Weight Hyaluronan Hydrogels. Applicant: ETH Zürich. Application EP. The sequence listing filed with the application follows.

SEQUENCE LISTING (39 sequences)

SEQ ID NO: 1 - protein, 8 aa, Homo sapiens
  MOD_RES 1: note = ACETYLATION
  MOD_RES 5: note = AMIDATION
FKGGERCG

SEQ ID NO: 2 - protein, 5 aa, Homo sapiens
  MOD_RES 1: note = ACETYLATION
  MOD_RES 5: note = AMIDATION
FKGGC

SEQ ID NO: 3 - protein, 8 aa, Homo sapiens
  MOD_RES 1: note = ACETYLATION
FKGGERCG

SEQ ID NO: 4 - protein, 5 aa, Homo sapiens
  MOD_RES 1: note = ACETYLATION
FKGGC

SEQ ID NO: 5 - protein, 5 aa, Homo sapiens
  MOD_RES 1: note = ACETYLATION
LKGGC

SEQ ID NO: 6 - protein, 4 aa, Homo sapiens
  MOD_RES 1: note = ACETYLATION
  SITE 1: note = Dopa (L-3,4-dihydroxyphenylalanine)
FKGC

SEQ ID NO: 7 - protein, 16 aa, Homo sapiens
  MOD_RES 1: note = ACETYLATION
  MOD_RES 16: note = AMIDATION
FKGGGPQGIWGQERCG

SEQ ID NO: 8 - protein, 16 aa, Homo sapiens
  MOD_RES 1: note = ACETYLATION
  MOD_RES 16: note = AMIDATION
FKGGGPQGIAGQERCG

SEQ ID NO: 9 - protein, 13 aa, Homo sapiens
  MOD_RES 1: note = ACETYLATION
FKGGGPQGIWGQC

SEQ ID NO: 10 - protein, 13 aa, Homo sapiens
  MOD_RES 1: note = ACETYLATION
FKGGGPQGIAGQC

SEQ ID NO: 11 - protein, 4 aa, Homo sapiens
  MOD_RES 1: note = ACETYLATION
  MOD_RES 4: note = AMIDATION
FKGC

SEQ ID NO: 12 - protein, 4 aa, Homo sapiens
  MOD_RES 1: note = ACETYLATION
FKGC

SEQ ID NO: 13 - protein, 4 aa, Homo sapiens
  MOD_RES 1: note = ACETYLATION
  MOD_RES 4: note = AMIDATION
LKGC

SEQ ID NO: 14 - protein, 4 aa, Homo sapiens
  MOD_RES 1: note = ACETYLATION
LKGC

SEQ ID NO: 15 - protein, 8 aa, Homo sapiens
NQEQVSPL

SEQ ID NO: 16 - protein, 4 aa, Homo sapiens
QQLG

SEQ ID NO: 17 - protein, 11 aa, Homo sapiens
GQLKHLEQQEG

SEQ ID NO: 18 - protein, 9 aa, Homo sapiens
NQEQVSPLC

SEQ ID NO: 19 - protein, 12 aa, Homo sapiens
NQEQVSPLERCG

SEQ ID NO: 20 - protein, 20 aa, Homo sapiens
NQEQVSPLGPQGIWGQERCG

SEQ ID NO: 21 - protein, 15 aa, Homo sapiens
NQEQVSPLGGGERCG

SEQ ID NO: 22 - protein, 12 aa, Homo sapiens
NQEQVSPLDRCG

SEQ ID NO: 23 - protein, 7 aa, Homo sapiens
  MOD_RES 1: note = ACETYLATION
  MOD_RES 5: note = AMIDATION
GQQQLGC

SEQ ID NO: 24 - protein, 10 aa, Homo sapiens
GQQQLGERCG

SEQ ID NO: 25 - protein, 10 aa, Homo sapiens
GQQQLGDRCG

SEQ ID NO: 26 - protein, 7 aa, Homo sapiens
GQQQLGC

SEQ ID NO: 27 - protein, 12 aa, Homo sapiens
GQLKHLEQQEGC

SEQ ID NO: 28 - protein, 15 aa, Homo sapiens
GQLKHLEQQEGERCG

SEQ ID NO: 29 - protein, 15 aa, Homo sapiens
GQLKHLEQQEGDRCG

SEQ ID NO: 30 - DNA, 19 bp, Homo sapiens
  source 1..19: mol_type = other DNA; note = fwd_primer_hRPL13a
aagtaccaggcagtgacag

SEQ ID NO: 31 - DNA, 20 bp, Homo sapiens
  source 1..20: mol_type = other DNA; note = rev_primer_hRPL13a
cctgtttccgtagcctcatg

SEQ ID NO: 32 - DNA, 19 bp, Homo sapiens
  source 1..19: mol_type = other DNA; note = fwd_primer_hCol1a1
cagccgcttcacctacagc

SEQ ID NO: 33 - DNA, 23 bp, Homo sapiens
  source 1..23: mol_type = other DNA; note = rev_hCol1a1
ttttgtattcaatcactgtcgcc

SEQ ID NO: 34 - DNA, 21 bp, Homo sapiens
  source 1..21: mol_type = genomic DNA; note = fwd_hCol2a1
ggaattcggtgtggacatagg

SEQ ID NO: 35 - DNA, 20 bp, Homo sapiens
  source 1..20: mol_type = other DNA; note = rev_hCol2a1
acttgggtcctttgggtttg

SEQ ID NO: 36 - DNA, 21 bp, Homo sapiens
  source 1..21: mol_type = other DNA; note = fwd_hCol10a1
attcctagtggctccaatgtg

SEQ ID NO: 37 - DNA, 21 bp, Homo sapiens
  source 1..21: mol_type = other DNA; note = rev_hCol10a1
gcctacctccatatgcatttt

SEQ ID NO: 38 - DNA, 21 bp, Homo sapiens
  source 1..21: mol_type = genomic DNA; note = fwd_hACAN
gaatgggaaccagcctatacc

SEQ ID NO: 39 - DNA, 22 bp, Homo sapiens
  source 1..22: mol_type = other DNA; note = rev_hACAN
tctgtactttcctctgttgctg